European Patent Specification EP 3 559 227 B1, published February 19, 2025. Title: Protease Variants and Uses Thereof. Applicant: Danisco US Inc. Babe, Lilia Marie Dankmeyer, Lydia Estell, David A. Goedegebuur, Frits Kaper, Thijs Mulder, Harm Pricelius, Sina. The sequence listing filed with the application follows.

SEQUENCE LISTING (22 sequences)

SEQ ID NO: 1 - protein, 269 aa, Bacillus lentus
AQSVPWGISRVQAPAAHNRGLTGSGVKVAVLDTGISTHPDLNIRGGASFVPGEPSTQDGNGHGTHVAGTIAALNNSIGVLGVAPSAELYAVKVLGASGSGSVSSIAQGLEWAGNNGMHVANLSLGSPSPSATLEQAVNSATSRGVLVVAASGNSGAGSISYPARYANAMAVGATDQNNNRASFSQYGAGLDIVAPGVNVQSTYPGSTYASLNGTSMATPHVAGAAALVKQKNPSWSNVQIRNHLKNTATSLGSTNLYGSGLVNAEAATR

SEQ ID NO: 2 - DNA, 1052 bp, Bacillus subtilis
gcaaaacgcggatcattggaagagacgaccgtacccgcagcatcaatgcctaaaataagcggatactctctgacgatattgcctcctgcttttccggccagaccatctttgtaattaatgccggaataagcaactttaatcaggacaccatccttcggcaaatcctctgttgatatggttttcacatggactgaaacatcatcggcatttttttctgcctgcaaggcttgaaataacgttgacattcggcacactccttttcatttatatcgtaaccgaagaacgttcaaaaaaccaaatcatcaagccgccattttcacttcgccggcacattgagacaataatggacaaatccggtatcctcttcatagccgttttgctcatacaagcttcttgccttccggttgtggtgctcagtctgaagtgttaaacattttgccccgttttgccctgcataatcctttgcggcagaaagcagccggccgccggctccctttgtacgcgcatgaggaacgacaaataagtcatttaatatgtatatccttttcattgacacagaagaaaacgttggatagagctgggtaaagcctatgaattctccattttcttctgctatcaaaataacagactcgtgattttccaaacgagctttcaaaaaagcctctgccccttgcaaatcggatgcctgtctataaaattcccgatattggttaaacagcggcgcaatggcggccgcatctgatgtctttgcttggcgaatgttcatcttatttcttcctccctctcaataattttttcattctatcccttttctgtaaagtttatttttcagaatacttttatcatcatgctttgaaaaaatatcacgataatatccattgttctcacggaagcacacgcgtcgctgataaacagctgacatcaactaaaagcttcattaaatactttgaaaaaagttgttgacttaaaagaagctaaatgttatagtaataaaacagaatagtcttttaagtaagtctactctgaatttttttaaaaggagagggtaaaga

SEQ ID NO: 3 - DNA, 87 bp, Bacillus subtilis
gtgagaagcaaaaaattgtggatcagcttgttgtttgcgttaacgttaatctttacgatggcgttcagcaacatgtctgcgcaggct

SEQ ID NO: 4 - DNA, 252 bp, Bacillus lentus
gctgaagaagcaaaagaaaaatatttaattggctttaatgagcaggaagctgtcagtgagtttgtagaacaagtagaggcaaatgacgaggtcgccattctctctgaggaagaggaagtcgaaattgaattgcttcatgaatttgaaacgattcctgttttatccgttgagttaagcccagaagatgtggacgcgcttgaactcgatccagcgatttcttatattgaagaggatgcagaagtaacgacaatg

SEQ ID NO: 5 - DNA, 810 bp, Bacillus lentus
gcgcaatcagtgccatggggaattagccgtgtgcaagccccagctgcccataaccgtggattgacaggttctggtgtaaaagttgctgtcctcgatacaggtatttccactcatccagacttaaatattcgtggtggcgctagctttgtaccaggggaaccatccactcaagatgggaatgggcatggcacgcatgtggccgggacgattgctgctttaaacaattcgattggcgttcttggcgtagcgccgagcgcggaactatacgctgttaaagtattaggggcgagcggttcaggttcggtcagctcgattgcccaaggattggaatgggcagggaacaatggcatgcacgttgctaatttgagtttaggaagcccttcgccaagtgccacacttgagcaagctgttaatagcgcgacttctagaggcgttcttgttgtagcggcatctggaaattcaggtgcaggctcaatcagctatccggcccgttatgcgaacgcaatggcagtcggagctactgaccaaaacaacaaccgcgccagcttttcacagtatggcgcagggcttgacattgtcgcaccaggtgtaaacgtgcagagcacatacccaggttcaacgtatgccagcttaaacggtacatcgatggctactcctcatgttgcaggtgcagcagcccttgttaaacaaaagaacccatcttggtccaatgtacaaatccgcaatcatctaaagaatacggcaacgagcttaggaagcacgaacttgtatggaagcggacttgtcaatgcagaagctgcaactcgttaa

SEQ ID NO: 6 - DNA, 254 bp, Bacillus amyloliquefaciens
tctagatacataaaaaaccggccttggccccgccggttttttattatttttcttcctccgcatgttcaatccgctccataatcgacggatggctccctctgaaaattttaacgagaaacggcgggttgacccggctcagtcccgtaacggccaagtcctgaaacgtctcaatcgccgcttcccggtttccggtcagctcaatgccgtaacggtcggcggcgttttcctgataccgggagacggcattcgtaatc

SEQ ID NO: 7 - DNA, 855 bp, Staphylococcus aureus
ttagtgacattagaaaaccgactgtaaaaagtacagtcggcattatctcatattataaaagccagtcattaggcctatctgacaattcctgaatagagttcataaacaatcctgcatgataaccatcacaaacagaatgatgtacctgtaaagatagcggtaaatatattgaattacctttattaatgaattttcctgctgtaataatgggtagaaggtaattactattattattgatatttaagttaaacccagtaaatgaagtccatggaataatagaaagagaaaaagcattttcaggtataggtgttttgggaaacaatttccccgaaccattatatttctctacatcagaaaggtataaatcataaaactctttgaagtcattctttacaggagtccaaataccagagaatgttttagatacaccatcaaaaattgtataaagtggctctaacttatcccaataacctaactctccgtcgctattgtaaccagttctaaaagctgtatttgagtttatcacccttgtcactaagaaaataaatgcagggtaaaatttatatccttcttgttttatgtttcggtataaaacactaatatcaatttctgtggttatactaaaagtcgtttgttggttcaaataatgattaaatatctcttttctcttccaattgtctaaatcaattttattaaagttcatttgatatgcctcctaaatttttatctaaagtgaatttaggaggcttacttgtctgctttcttcattagaatcaatccttttttaaaagtcaatattactgtaacataaatatatattttaaaaatatcccactttatccaattttcgtttgt

SEQ ID NO: 8 - DNA, 994 bp, artificial sequence
  3' flanking region
tcagccttattctcctgataacgcgagacagcattagaaaaaggcgtaaccgcaaagctcaaaacagaaaacaaaagcaataacagcggaagtgccgcaagatcatgccgcccttctaaatgaaacatgctgcgggttaggcgaaccgtccgcttgtaaagcttatcaatgacataaaatccggcgagcgacacgagcaaatagccagccagaccgatgtaaacgtgcttcatgacataatggcccatttcgtggcccataataaacagaatttctgaatcgtcaagtttgttcagcgtcgtatcccacaatacaatccgtttattggccccaattcctgtaacataggcattcagcgcatttgttttttctgacatgttcacttcatatacatggtcagccggaatattggcttcatctgccagctctaaaattttgctttcaagctctttgtttttcagcggataaaaatcattgtataaaggatcgataatgaccggctgaataaaaaacagaaacagcgaaaacggcactgttaacagccaggcgtataaccaccattttttttcatgccttttgatcagccaataaaaaacgagaacgcaaagcgtaaagattggaaagctgatccaaaagctgataacctgatccttagcccagctggccgttgtctgtgtggaaatgttatagtcaagcgatacttgatagcctatccaatctaaaggcagcgtcaccaatgttgtaatcagcgaaagcacaaacacaaaaccaacggtctgcaaaaaccgaaaaggcacggccgcttcgatccatttcttgattttctttgaaacaccgctgacaagcagaacaaaaaacagaaaccaatcaagtggtaccccgataaaaaataaaaaattcttgacattcgaatactgctcggccactgccaactcagacggcttcatgaaagaagccggatcagcctgcgtccctttcacggcttccggtattg

SEQ ID NO: 9 - protein, 29 aa, Bacillus subtilis
VRSKKLWISLLFALTLIFTMAFSNMSAQA

SEQ ID NO: 10 - protein, 84 aa, Bacillus lentus
AEEAKEKYLIGFNEQEAVSEFVEQVEANDEVAILSEEEEVEIELLHEFETIPVLSVELSPEDVDALELDPAISYIEEDAEVTTM

SEQ ID NO: 11 - protein, 269 aa, Bacillus gibsonii
QQTVPWGITRVQAPAVHNRGITGSGVRVAILDSGISAHSDLNIRGGASFVPGEPTTADLNGHGTHVAGTVAALNNSIGVIGVAPNAELYAVKVLGANGSGSVSGIAQGLEWAATNNMHIANMSLGSDFPSSTLERAVNYATSRDVLVIAATGNNGSGSVGYPARYANAMAVGATDQNNRRANFSQYGTGIDIVAPGVNVQSTYPGNRYVSMNGTSMATPHVAGAAALVKQRYPSWNATQIRNHLKNTATNLGNSSQFGSGLVNAEAATR

SEQ ID NO: 12 - DNA, 810 bp, Bacillus gibsonii
caacaaacagtgccatggggaattactcgtgtgcaagccccagctgttcataaccgtggaattacaggttctggtgtaagagttgctatcctcgattcaggtatttccgcacatagcgacttaaatattcgtggtggcgcaagctttgtaccaggggaaccaacgactgctgatttaaatgggcatggcacgcatgtggctgggacggtagctgctttaaacaattcgattggcgttattggcgtagcaccgaatgcggaactatacgctgttaaagtattaggggcgaatggtagcggttcggtcagcgggattgcccaaggattggaatgggcagcaacaaataacatgcacattgctaatatgagtttaggaagcgattttccaagttctacacttgagcgtgctgttaattatgcgacttctagagatgttcttgttattgcggcaactgggaataacggttctggctcagtaggctatccggcccgttatgcgaacgcaatggcagtcggagctactgaccaaaacaacagacgcgccaacttttcacagtatggcacggggattgacattgtcgcaccaggtgtaaacgtgcagagcacatacccaggtaaccgttatgtgagcatgaacggtacatcgatggctactcctcatgttgcaggtgcagcagcccttgttaaacaacgctatccatcttggaatgcgactcaaatccgcaatcatctaaagaatacggcaacgaatttaggaaactcttcacaatttggaagcggacttgtcaatgcagaagcggcaacacgctaa

SEQ ID NO: 13 - protein, 269 aa, Bacillus gibsonii
QQTVPWGITRVQAPTVHNRGITGSGVKVAILDTGIAQHSDLTIRGGASFVPGESTTADLNGHGTHVAGTVAALNNSIGVIGVAPSADLYAVKVLGANGRGSVSGIAQGLEWAATNNMHIANMSLGSDAPSTTLERAVNYATSRGVLVIAATGNNGTGSIGYPARYANAMAVGATDQNNRRASFSQYGTGIDIVAPGVGIQSTYLNNSYASMPGTSMATPHVAGVAALVKQKNPSWNATQIRNHLKNTATNLGNSSQFGSGLVNADAATR

SEQ ID NO: 14 - DNA, 810 bp, Bacillus gibsonii
caacaaacagtgccatggggaattactcgtgtgcaagccccaacagttcataaccgtggaattacaggttctggtgtaaaagttgctatcctcgatacaggtattgcacaacattcagacttaacaattcgtggtggcgcaagctttgtaccaggggaatcaacgacagctgatttaaatgggcatggcacgcatgtggctgggacggtagctgctttaaacaattcgattggcgttattggcgtagcaccgtcagcggatctatacgctgttaaagtattaggggcgaatggtagaggttcggtcagcgggattgcccaaggattggaatgggcagcaacaaataacatgcacattgctaatatgagtttaggatcagatgcaccaagtacaacacttgagcgtgctgttaattatgcgacttctagaggcgttcttgttattgcggcaactgggaataacggtacaggctcaattggctatccggcccgttatgcgaacgcaatggcagtcggagctactgaccaaaacaacagacgcgcctcattttcacagtatggcacggggattgacattgtcgcaccaggtgtaggcattcagagcacatacctgaataactcatatgcaagcatgccgggtacatcgatggctactcctcatgttgcaggtgttgcagcccttgttaaacaaaaaaatccatcttggaatgcgactcaaatccgcaatcatctaaagaatacggcaacgaatttaggaaactcttcacaatttggaagcggacttgtcaatgcagatgcggcaacacgctaa

SEQ ID NO: 15 - protein, 274 aa, Bacillus licheniformis
AQTVPYGIPLIKADKVQAQGFKGANVKVAVLDTGIQASHPDLNVVGGASFVAGEAYNTDGNGHGTHVAGTVAALDNTTGVLGVAPSVSLYAVKVLNSSGSGSYSGIVSGIEWATTNGMDVINMSLGGASGSTAMKQAVDNAYARGVVVVAAAGNSGSSGNTNTIGYPAKYDSVIAVGAVDSNSNRASFSSVGAELEVMAPGAGVYSTYPTNTYATLNGTSMASPHVAGAAALILSKHPNLSASQVRNRLSSTATYLGSSFYYGKGLINVEAAAQ

SEQ ID NO: 16 - DNA, 822 bp, Bacillus licheniformis
gcgcaaaccgttccttacggcattcctctcattaaagcggacaaagtgcaggctcaaggctttaagggagcgaatgtaaaagtagccgtcctggatacaggaatccaagcatctcatccggacttgaacgtagtcggcggagcgagctttgtggctggcgaagcatataacaccgacggcaacggacacggcacacatgttgccggtacagtagctgcgcttgacaatacaacgggtgtattaggcgttgcgccaagcgtatccttgtacgcggttaaagtactgaactcaagcggaagcggatcatacagcggcattgtaagcggaatcgagtgggcgacaacaaacggcatggatgttatcaatatgagccttgggggagcatcaggctcgacagcgatgaaacaggcagtcgacaatgcatacgcaagaggggttgtcgttgtagcagcagctgggaacagcggatcttcaggaaacacgaatacaattggctatcctgcgaaatacgattctgtcatcgctgttggcgcggtagactctaacagcaacagagcttcattttccagtgtgggagcagagcttgaagtcatggctcctggcgcaggcgtatacagcacttacccaacgaacacttatgcaacattgaacggaacgtcaatggcttctcctcatgtagcgggagcagcagctttgatcttgtcaaaacatccgaacctttcagcttcacaagtccgcaaccgtctctccagcacggcgacttatttgggaagctccttctactatgggaaaggtctgatcaatgtcgaagctgccgctcaa

SEQ ID NO: 17 - protein, 275 aa, Bacillus amyloliquefaciens [sequence omitted]

SEQ ID NO: 18 - DNA, 828 bp, Bacillus amyloliquefaciens
gcgcagtccgtgccttacggcgtatcacaaattaaagcccctgctctgcactctcaaggctacactggatcaaatgttaaagtagcggttatcgacagcggtatcgattcttctcatcctgatttaaaggtagcaggcggagccagcatggttccttctgaaacaaatcctttccaagacaacaactctcacggaactcacgttgccggcacagttgcggctcttaataactcaatcggtgtattaggcgttgcgccaagcgcatcactttacgctgtaaaagttctcggtgctgacggttccggccaatacagctggatcattaacggaatcgagtgggcgatcgcaaacaatatggacgttattaacatgagcctcggcggaccttctggttctgctgctttaaaagcggcagttgataaagccgttgcatccggcgtcgtagtcgttgcggcagccggtaacgaaggcacttccggcagctcaagcacagtgggctaccctggtaaatacccttctgtcattgcagtaggcgctgttgacagcagcaaccaaagagcatctttctcaagcgtaggacctgagcttgatgtcatggcacctggcgtatctatccaaagcacgcttcctggaaacaaatacggggcgtacaacggtacgtcaatggcatctccgcacgttgccggagcggctgctttgattctttctaagcacccgaactggacaaacactcaagtccgcagcagtttagaaaacaccactacaaaacttggtgattctttctactatggaaaagggctgatcaacgtacaggcggcagctcagtaa

SEQ ID NO: 19 - DNA, 228 bp, Bacillus licheniformis
gctcaaccggcgaaaaatgttgaaaaggattatattgtcggatttaagtcaggagtgaaaaccgcatctgtcaaaaaggacatcatcaaagagagcggcggaaaagtggacaagcagtttagaatcatcaacgcggcaaaagcgaagctagacaaagaagcgcttaaggaagtcaaaaatgatccggatgtcgcttatgtggaagaggatcatgtggcccatgccttg

SEQ ID NO: 20 - protein, 76 aa, Bacillus licheniformis
AQPAKNVEKDYIVGFKSGVKTASVKKDIIKESGGKVDKQFRIINAAKAKLDKEALKEVKNDPDVAYVEEDHVAHAL

SEQ ID NO: 21 - DNA, 231 bp, Bacillus amyloliquefaciens
gcagggaaatcaaacggggaaaagaaatatattgtcgggtttaaacagacaatgagcacgatgagcgccgctaagaagaaagatgtcatttctgaaaaaggcgggaaagtgcaaaagcaattcaaatatgtagacgcagcttcagctacattaaacgaaaaagctgtaaaagaattgaaaaaagacccgagcgtcgcttacgttgaagaagatcacgtagcacatgcgtac

SEQ ID NO: 22 - protein, 77 aa, Bacillus amyloliquefaciens
AGKSNGEKKYIVGFKQTMSTMSAAKKKDVISEKGGKVQKQFKYVDAASATLNEKAVKELKKDPSVAYVEEDHVAHAY